European Patent Application EP 4 470 541 A1, published December 4, 2024. Title: OVARIAN ANTI-AGING PHARMACEUTICAL COMPOSITION AND USE THEREOF. Applicant: MitoImmune Therapeutics Inc. Application KR PCT/KR2023/001264, filed January 27, 2023. The sequence listing filed with the application follows.

SEQUENCE LISTING (10 sequences)

SEQ ID NO: 1 - RNA, 22 nt, Synthetic construct
  source 1..22: mol_type = other RNA
ggacttctatgacctgtacgga

SEQ ID NO: 2 - RNA, 21 nt, Synthetic construct
  source 1..21: mol_type = other RNA
cgagcagttcagtgggtactt

SEQ ID NO: 3 - RNA, 22 nt, synthetic construct
  source 1..22: mol_type = other RNA
atctcagccgtgatcttgttct

SEQ ID NO: 4 - RNA, 23 nt, synthetic construct
  source 1..23: mol_type = other RNA
accatacaaaaacaggacagcat

SEQ ID NO: 5 - RNA, 21 nt, synthetic construct
  source 1..21: mol_type = other RNA
cccaagatgcgactgttcttc

SEQ ID NO: 6 - RNA, 19 nt, synthetic construct
  source 1..19: mol_type = other RNA
gtcccttgacctcgggaga

SEQ ID NO: 7 - RNA, 19 nt, synthetic construct
  source 1..19: mol_type = other RNA
agaaaagctatgagacgcc

SEQ ID NO: 8 - RNA, 19 nt, synthetic construct
  source 1..19: mol_type = other RNA
aggacctcaaaagccaatc

SEQ ID NO: 9 - RNA, 19 nt, synthetic construct
  source 1..19: mol_type = other RNA
acttcaactgacttggtgg

SEQ ID NO: 10 - RNA, 19 nt, synthetic construct
  source 1..19: mol_type = other RNA
aaatcctgttcttcctggc